European Patent Specification EP 2 814 966 B1, published June 3, 2026. Title: Improving drought resistance in plants: UPL4. Applicant: Keygene N.V. The sequence listing filed with the application follows.

SEQUENCE LISTING (12 sequences)

SEQ ID NO: 1 - DNA, 4509 bp, Arabidopsis thaliana
atggagaacagaggccagaaacgaatggaggttgtggaagagttacctgctgataagagagcttgtaactctcaggattttagaccaagcacatccggatcatctgttcaagctcaagctaatgatacgaatccaggacatgaaaacgttgacgctgatatggatacttcttcatctgcttcgccttcgagtcgatcagatgaagaagaacaggaagagcaggataaggaggattcggactatggatcttgcgattctgatgaggaagatccgaggcagagggtgcttcaggattaccagaggcagagatcatctggtgatcatgggaaattgaagtctcttttgttgaatttgactggagaaactgatccttctggacagttatccaggctcactgagttatgtgaagtgttgtcattttctactgaagaatcgctgtccagtgttatggccaacatgctatcaccggtgcttgtaaagttagctaagcatgagaacaatgcagatattatgctcctcgcaattagagctattacttatttgtgtgatgtttatccgccgtcagtagaattccttgtaagacatgataccattcctgctctctgccaaagacttttgactattgagtacttggacgttgctgagcagtgtttgcaagcacttgagaaaatatcccgagatgagccggtagcctgcttgaatgctggagcaattatggcagtgctttcgtttattgatttcttctcaacaagcatacagagagtcgcaatttctactgtggtcaatatatgtaagcagctttcttctgagtctccctcgcctttcatggatgctgttccaatattatgcactcttcttcaatatgaagatcgacagctggtcgagaatgtggctatttgcttgacaaaaatagcagatcaagccagtgagtcaccggcaatgttggatcaactgtgtaggcatggactaattaatgaatcaacacatctcttaaacttgaatagccgcactaccctatctcaacctgtctacaatggtgtgattggaatgctaagaaaactatcttctggttcagctttagctttcagaacgttatatgagcttaacattggctacagtttaaaagaaatcatgtccacgtatgacatttctcattcagtgtcttctacacatcctatcaatgcatgttctaatcaggtgcatgaagtcctgaagttggtgattgagcttcttccagcttcacccgtagaggataatcagctggcatcggaaaaggaaagttttctcgtcaatcagcctgatcttttgcaacaatttggaagagacatgcttcctgtcatgattcaggtgctaaactctggagctaacgtatatgtttcttatggttgcctatcagcaattcacaagctgacttgcttgagtaagtccggtgatattgtcgagttactgaagaacaccaacatgtcaagtgttttggctggcattctgtcaaggaaggatcatcatgtaattgtagtagcactacaggttgcggaagtgcttcttgagaaatacagagatacttttttgaattcttttataaaggaaggtgtttttttcgcgattgaagcactcttaagttctgatagagggcaacaaaatcagggatcagctgacctttcacaaaagcctgttacaaaagagattgtgaaatgcttgtgccaatcttttgaaagatcgctatcctcttcttcacaaacttgtaagattgaaaaggattctgtctacgttcttgcaacacgtatcaaggagggtttctttggacctgaggtattcaactctgagaaaggcttgacagatgtcctccaaaacctcaagaacttgtcggtagcacttagcgagttgatgactgtacccattgatgcgcatgtcctgcatgatgagaaattcttctcaatatggaaccaaatcatggaaaggctgaatggaagggaatctgtgtccacttttgaattcattgagagcggagttgtaaagtcactggcaagttatctttctaatggactctatcaaaggaaacttagcaaagggggtcctgaatgtgatagtttaccatttattggtaagagatttgaggtgttcacaagattgctttggtctgatggagaggcaacttcatccttgttaatacagaagctccaaaattccctttcttctttggaaaacttcccaattgtcctaagccaatttttgaagcagaagaactcatttgcggctattccaaatgggcgttgcactagttatccatgcctaaaagttcgttttctgaaagcagagggggagacttctttgcgtgattactcccaagactttgtcactgttgacccactttgctatttggatgctgtcgatcaatacttgtggcctaaagttaatatagaacctatagattctgtggaagcaaaagatcaagctatagaatgtcaatcttctcaattgcagtcaacttcgatatcttgtcaagctgaaagctcaagtcctatggagattgacagtgagtcttctgatgcgtctcagttgcagggatctcaagtggaagatcagacgcaacttccaggacaacagaatgcttcctcctctgaaacctcctctgaaaaagaggatgcggtacctagacttttgtttcgtctcgaagggcttgaactagaccgttctttgacagtatatcaggcgattctcttgcacaaactaaaatcagaaagtgaagcaaccaacgattcgaagctgagtggaccccacaacatcacttatgaaaggtctgcacaacttggggattctcgtgaaaatctgtttccacctggatctatggaagatgatgagtatcgcccgttcttgtcctatttgtttactcatagacttgctttgcgcctgaaggggtcaagtcatcctccgtatgacatattgtttcttcttaagagtctggagggcatgaacagatttctctttcacctgatttctcttgaacggattaatgcttttggtgaaggtaggctagagaatttggatgatctgagggtacaagttcgtcctgtgccacattctgaatttgttagcagtaagcttacagagaagttagagcagcagcttcgtgattcttttgctgtgtcaacctgcggtctgccaccatggtttaatgatctaatggattcatgtccgtgtttatttagttttgaagccaagtctaaatacttccgacttgcagcctttggttcacagaaaatccgtcatcatccacagcaccttagcagttcaaatgttcatggcgaagcgcgcccagtgactggtagtttacctcgtaaaaagttcttagcttgccgtgaaaacattctagagtctgctgccaaaatgatggagttatatggaaaccagaaggtggtcattgaggttgaatacagtgaagaagtcgggactggtcttgggccaacactggagttctatacgcttgtcagtagggcatttcaaaatcccgatcttggtatgtggagaaatgattgtagttttattgttggaaagccagtcgaacactcgggagttttggcatcttcttcaggactctttccacgcccttggtcaggtacatcaactacgtcagatgtgctgcagaaatttgtcctcttggggacagtggtagcaaaggctttacaagatggacgagtcttagaccttccactttccaaagccttctacaaattaattctcggacaggagttgagttcatttgacatccacttcgttgaccctgaactttgtaaaacactggtggaattgcaagctctggtacgtaggaaaaagcttttcgctgaagcacatggtgattccggagcagccaagtgtgatttaagtttccatggaacaaagattgaggacctttgtcttgaatttgcattgcctggctacacggattatgatctcgctccctattctgcaaatgatatggtaaatttggataacctcgaggaatatatcaagggtattgtcaatgccacagtatgtaatgggatccaaaaacaagtggaagcatttcggtctggatttaatcaggttttctctattgaacatcttcggatattcaacgaagaggagctggaaactatgctgtgtggagaatgtgatctctttagtatgaatgaagtcttggatcacatcaagtttgatcatggatatacttctagcagcccaccagttgaatatttattgcagattctgcatgagtttgatagggagcaacaacgagcctttttgcaatttgtaacaggatctccccggttacctcatggtggtttggcgtctctcagtcccaaactaacaatcgtccgcaagcatggtagcgattcttcagatactgacctccctagtgtgatgacatgcgccaattatctgaagcttcctccttattcatccaaagagaagatgaaggagaagctgatttatgccataacggaaggtcaaggttccttccatctctcttaa

SEQ ID NO: 2 - protein, 1502 aa, Arabidopsis thaliana
MENRGQKRMEVVEELPADKRACNSQDFRPSTSGSSVQAQANDTNPGHENVDADMDTSSSASPSSRSDEEEQEEQDKEDSDYGSCDSDEEDPRQRVLQDYQRQRSSGDHGKLKSLLLNLTGETDPSGQLSRLTELCEVLSFSTEESLSSVMANMLSPVLVKLAKHENNADIMLLAIRAITYLCDVYPPSVEFLVRHDTIPALCQRLLTIEYLDVAEQCLQALEKISRDEPVACLNAGAIMAVLSFIDFFSTSIQRVAISTVVNICKQLSSESPSPFMDAVPILCTLLQYEDRQLVENVAICLTKIADQASESPAMLDQLCRHGLINESTHLLNLNSRTTLSQPVYNGVIGMLRKLSSGSALAFRTLYELNIGYSLKEIMSTYDISHSVSSTHPINACSNQVHEVLKLVIELLPASPVEDNQLASEKESFLVNQPDLLQQFGRDMLPVMIQVLNSGANVYVSYGCLSAIHKLTCLSKSGDIVELLKNTNMSSVLAGILSRKDHHVIVVALQVAEVLLEKYRDTFLNSFIKEGVFFAIEALLSSDRGQQNQGSADLSQKPVTKEIVKCLCQSFERSLSSSSQTCKIEKDSVYVLATRIKEGFFGPEVFNSEKGLTDVLQNLKNLSVALSELMTVPIDAHVLHDEKFFSIWNQIMERLNGRESVSTFEFIESGVVKSLASYLSNGLYQRKLSKGGPECDSLPFIGKRFEVFTRLLWSDGEATSSLLIQKLQNSLSSLENFPIVLSQFLKQKNSFAAIPNGRCTSYPCLKVRFLKAEGETSLRDYSQDFVTVDPLCYLDAVDQYLWPKVNIEPIDSVEAKDQAIECQSSQLQSTSISCQAESSSPMEIDSESSDASQLQGSQVEDQTQLPGQQNASSSETSSEKEDAVPRLLFRLEGLELDRSLTVYQAILLHKLKSESEATNDSKLSGPHNITYERSAQLGDSRENLFPPGSMEDDEYRPFLSYLFTHRLALRLKGSSHPPYDILFLLKSLEGMNRFLFHLISLERINAFGEGRLENLDDLRVQVRPVPHSEFVSSKLTEKLEQQLRDSFAVSTCGLPPWFNDLMDSCPCLFSFEAKSKYFRLAAFGSQKIRHHPQHLSSSNVHGEARPVTGSLPRKKFLACRENILESAAKMMELYGNQKVVIEVEYSEEVGTGLGPTLEFYTLVSRAFQNPDLGMWRNDCSFIVGKPVEHSGVLASSSGLFPRPWSGTSTTSDVLQKFVLLGTVVAKALQDGRVLDLPLSKAFYKLILGQELSSFDIHFVDPELCKTLVELQALVRRKKLFAEAHGDSGAAKCDLSFHGTKIEDLCLEFALPGYTDYDLAPYSANDMVNLDNLEEYIKGIVNATVCNGIQKQVEAFRSGFNQVFSIEHLRIFNEEELETMLCGECDLFSMNEVLDHIKFDHGYTSSSPPVEYLLQILHEFDREQQRAFLQFVTGSPRLPHGGLASLSPKLTIVRKHGSDSSDTDLPSVMTCANYLKLPPYSSKEKMKEKLIYAITEGQGSFHLS

SEQ ID NO: 3 - DNA, 5667 bp, Arabidopsis thaliana
atggaaactcggagccgcaagcgggcggaggcgacctcagctgccccatcttcttcttcttcttctcctcctcctcctccctctgcctctggtcccaccacccgcagcaaacgcgctcgtctttcttcttcttcttcttcctcacttgcccccactcctccttcttcctccaccaccacccgctctcgttcttctcgctctgccgccgccgctgctcccatggacacctccaccgactcttctggatttcgccgaggcggacgtggtaacaggggaaacaacaacgataattctgacaaaggtaaggagaaggaacatgacgttaggattagggagcgtgaaagagaaagagaccgagccagagaacaactcaacatggatgctgccgccgccgctgctaggagcgctgacgaggatgacgacaatgacagtgaggatggcaacggcggtttcatgcatcctaacatgagctctgcgagcagtgctttacaaggcttgctcaggaagctcggtgctggattggatgacttgcttccttcttccggtatcggctctgcttcttcctcccacttgaatggaaggatgaagaagattctctctggcttgcgcgctgaaggagaagagggaaaacaggtcgaggctttaacccagctttgtgagatgttatccattgggaccgaagactcgcttagcaccttctctgttgattccttcgtcccagttcttgtcggtctacttaaccatgaaagcaatcccgacattatgcttcttgctgccagggctcttacccatctatgtgatgtcttgccgtcttcttgtgctgctgttgtacattacggggcagtttcatgcttggtggccagattgctaaccatagaatacatggacttggcggaacagtctctgcaagctctcaaaaagatatctcaggagcacccaactgcctgtttgcgagctggtgctcttatggctgtgctctcgtatctggatttcttctccactggtgttcagcgcgtagcactatctactgctgccaacatgtgcaagaaactaccttctgatgcatctgattatgttatggaagctgtacctttgctgacaaacctacttcagtatcatgattcgaaggttttggaatatgcttctatctgtctgactcgaattgctgaagcatttgcaccgtatcccgagaaattagatgaattatgtaaccatggcctggtgacgcaagctgcgtctcttatttccacgagcaattcaggaggtgggcaagcatctcttagtgtgtcaacatacacggggttaatccgattactttctacctgtgcgagcgggtcacctcttggattcaggacattacttcttcttggtattagtagcattcttaaggatattctgttgggttctggggtctctgctaatgcatctgtatccccagcactgagccggcctgcagatcagatttatgagatagtcaacctagcgaatgagctcctccctccattgccagaaggagttatctctcttcctactagcacaaacgctcttgtgaaaggttcatgccaaaagaaatctagtccaagtacttcaggaaaacaagaagatattctaaaaatttcaccaagagaaaaattacttggtgatcaacctgaacttctgcagcagtttggattggatcttcttccagttttagtgcagatctatggttctagtgtcaatggtacgattcgccataaatgtctctcagtcattggaaagttgatgtatttcagcagttcagaaatgattcaatctctaattggtgacacaaatatttcgagcttcttggctggtgtcttggcatggaaagacccacaggtcttggttcctgctctacaagttgcagagattttgatggaaaagcttcctgaaacattctcgaaagtgtttgtgagggaaggggtagtccatgctgtagatcaacttgtcttggttggtaaaccatcccatgcctcacctactgataaggacaatgactgtgtacccggatctgcacgatctaggcgttatagacggcgcagtagtaatgccaattccgatggaaaccagtcggaagagcctaagaatcctgcgtcccttaccataggggcaaaccataattcccttgatactcctacagctagcttcatgctaagggaaacagttagttcctgcgccaaagcattcaaagacaagtacttcccgtctgatggtggggatgttgatgttggagttacagatgatcttttacatctgaagaatctttgcacgaagctaactgctggtatagatgatcataaagtgaaaggaaagggaaaatctaaagcctctgggccattccttggcgatttctctgctagcaaggaagagtacttgattggtgtcatttctgagatacttggcgagataagtaaaggggatggtgtctcaacttttgagtttattggcagtggtgtggttgcagcattgcttaactatttttcttgtggatacttttccaaagagaagatctccgaacttaatttgcccaaacttcgccaggagggactcagaaggtttaaagcttttctagaagtcgctcttccttttgatggtaatgagggaaaggtccctcctatgacagttttgattcagaaacttcaaaatgctttatcgtcactggagcgctttcctgttgtccttagccatccctcaaggtcactaagtggaagtgctcggctctcctcgggtttgagtgctttggcacatcctttaaagttgcgattatgccgagcatctggagagaaaacactacgtgattactcctccaatattgtacttatagatccattggcaagcttagcagcagtggaggaatttctgtggccccgagttcaacggagtgaatctgctctgaagccggcagcgcctattggcaatacagagccaggcacgttacctagcggtgctggtgtttcatcaccatcttcgtcaactccagcttcaaccactcgtcgtcattcttctagatctcgatcggcaattaacatcggtgatacttcaaagaaagatcctgtgcatgagaaaggtaccagctcatcgaaaggaaaaggtaaaggcgttatgaaaccggctcaggcggataaggggcctcaaacaaggagcaatgctcaaaagagagctgttcttgacaaagatactcaaatgaaaccagctagcggagactccagttctgaggatgaggaattggaaatatccccagtcgacattgatgatgccttggtgattgaagaggatgacatttctgatgatgaagatgatgataatgaagatgttttggatgacagtcttcccatgtgcacgcctgataaagtccatgatgtgaaattggcggactcagtggatgatgatggtctagcaaccagcggccgacaaatgaatccagcttctggaggcactagtggagccgcagcagcaagggcatctgattctattgatactggcattgggaattcctatggttctagaggtgcactctcctttgctgctgcagcgatggctgggcttggagctgccagtggtagaggtatcaggggaagtagggacttgcatggacgtaccctaaatcgaagttcagatgagccctctaagttgatatttactgcggcaggaaaacaacttagtaggcatttgacgatttatcaggctgtacagcgacaacttatgctagatgaagatgatgatgacaggtttggtggcagtgatctagtctcaagtgatggaagcagattcaatgatatttacaccatcatgtaccagaggccagacagccaagtgaataggttgtctgttggtggagcaagttctaccacaccgtcaaaatccacgaaatctgctactaccaattccagtgtagaatctcagtcacatagggcatctcttttggatagtatcttacaaggggagcttccatgcgaccttgagaagtcgaattctacatataatgttctggcactgttacgtgtattagagggtttaaatcagctttgccctcgtttaagagcccaaactctttccgatcgttttgcagagggtaaaattacaagtctagatgatctgagtacaactgctgctaaggttcctcttgatgaatttgtcaatagcaaacttacacccaaattggctcgacaaatccaggatgcgcttgctttgtgcagtggaagtcttccctcttggtgctaccagttgactagagcatgcccatttttgtttccgtttcaaacccggagacagtatttctactcgactgcttttgggttgtctcgtgcattgaatcgtttgcagcagcagcaaggtgctgacggcagtgggtctacaaatgaacgagagatgagaatagggagattgcagcgccagaaagtccgtgtatcccgaaataggatattagattctgctgcaaaagttatggagatgtattctagccagaaagctgtgcttgaagtagaatattttggtgaagttggtactggtctaggccctacccttgagttttacacacttctaagccatgatctgcaaaaggcttccctagggatgtggagatcaagttctggtgacaaggtatctatgcaaattggtagagatgagattgaagacggaaaaccatctgcagctaacagagatatagttctggcaccacttggattgtttcctcggccttggccctcaacagctgacatatctgaaggtggtcagtttcataaagtcattgaatatttccgccttttagggcgtgtgatggccaaagcacttcaagatggacggctattggacgtcccattgagtacagcgttttataaacttattcttggtcaagagcttgatttgcatgatattgtattatttgacgctgaacttggcaagaccttgcaagagctgcgtgttgttgttgcccgcaagcactatctggagggagtaggtggtgacaatagcagcacgatttctgatttatgtttacgtggatgccgaatagaagatctctccttggaattcacgctacctggctatcctgagtacatcctgagatcaggagatgaaattgttgatattactaatcttgaggagtatatatcccttgtcgttgatgctactgtcaagagaggagtcactcggcagatcgaagccttcagatctggattcaatcaggtgtttgacataacatctctacaaatattcaccccttctgagctggactatttgctgtgtggtcgtagagagttgtgggaggtggagactcttgctgaacatatcaaatttgatcatgggtataatgccaaaagtccggcaatcattaacttactggagatcatgggagaacttacagcagatcagcagagggctttctgccaatttgtaactggagctcctaggcttcctcctggtggcttagctgttctgaacccaaagcttacgattgtgagaaagcactcatcgacctcaagtgcagcagccaacggagcaggggcttcggagacagcagatgatgatttgcccagtgtcatgacttgcgcaaactaccttaaactccctccttattctacaaaggaaatcatgtacaagaaactgctctacgccatcaacgaagggcaaggatcgttcgacctctcataa

SEQ ID NO: 4 - protein, 1888 aa, Arabidopsis thaliana
METRSRKRAEATSAAPSSSSSSPPPPPSASGPTTRSKRARLSSSSSSSLAPTPPSSSTTTRSRSSRSAAAAAPMDTSTDSSGFRRGGRGNRGNNNDNSDKGKEKEHDVRIRERERERDRAREQLNMDAAAAAARSADEDDDNDSEDGNGGFMHPNMSSASSALQGLLRKLGAGLDDLLPSSGIGSASSSHLNGRMKKILSGLRAEGEEGKQVEALTQLCEMLSIGTEDSLSTFSVDSFVPVLVGLLNHESNPDIMLLAARALTHLCDVLPSSCAAVVHYGAVSCLVARLLTIEYMDLAEQSLQALKKISQEHPTACLRAGALMAVLSYLDFFSTGVQRVALSTAANMCKKLPSDASDYVMEAVPLLTNLLQYHDSKVLEYASICLTRIAEAFAPYPEKLDELCNHGLVTQAASLISTSNSGGGQASLSVSTYTGLIRLLSTCASGSPLGFRTLLLLGISSILKDILLGSGVSANASVSPALSRPADQIYEIVNLANELLPPLPEGVISLPTSTNALVKGSCQKKSSPSTSGKQEDILKISPREKLLGDQPELLQQFGLDLLPVLVQIYGSSVNGTIRHKCLSVIGKLMYFSSSEMIQSLIGDTNISSFLAGVLAWKDPQVLVPALQVAEILMEKLPETFSKVFVREGVVHAVDQLVLVGKPSHASPTDKDNDCVPGSARSRRYRRRSSNANSDGNQSEEPKNPASLTIGANHNSLDTPTASFMLRETVSSCAKAFKDKYFPSDGGDVDVGVTDDLLHLKNLCTKLTAGIDDHKVKGKGKSKASGPFLGDFSASKEEYLIGVISEILGEISKGDGVSTFEFIGSGVVAALLNYFSCGYFSKEKISELNLPKLRQEGLRRFKAFLEVALPFDGNEGKVPPMTVLIQKLQNALSSLERFPVVLSHPSRSLSGSARLSSGLSALAHPLKLRLCRASGEKTLRDYSSNIVLIDPLASLAAVEEFLWPRVQRSESALKPAAPIGNTEPGTLPSGAGVSSPSSSTPASTTRRHSSRSRSAINIGDTSKKDPVHEKGTSSSKGKGKGVMKPAQADKGPQTRSNAQKRAVLDKDTQMKPASGDSSSEDEELEISPVDIDDALVIEEDDISDDEDDDNEDVLDDSLPMCTPDKVHDVKLADSVDDDGLATSGRQMNPASGGTSGAAAARASDSIDTGIGNSYGSRGALSFAAAAMAGLGAASGRGIRGSRDLHGRTLNRSSDEPSKLIFTAAGKQLSRHLTIYQAVQRQLMLDEDDDDRFGGSDLVSSDGSRFNDIYTIMYQRPDSQVNRLSVGGASSTTPSKSTKSATTNSSVESQSHRASLLDSILQGELPCDLEKSNSTYNVLALLRVLEGLNQLCPRLRAQTLSDRFAEGKITSLDDLSTTAAKVPLDEFVNSKLTPKLARQIQDALALCSGSLPSWCYQLTRACPFLFPFQTRRQYFYSTAFGLSRALNRLQQQQGADGSGSTNEREMRIGRLQRQKVRVSRNRILDSAAKVMEMYSSQKAVLEVEYFGEVGTGLGPTLEFYTLLSHDLQKASLGMWRSSSGDKVSMQIGRDEIEDGKPSAANRDIVLAPLGLFPRPWPSTADISEGGQFHKVIEYFRLLGRVMAKALQDGRLLDVPLSTAFYKLILGQELDLHDIVLFDAELGKTLQELRVVVARKHYLEGVGGDNSSTISDLCLRGCRIEDLSLEFTLPGYPEYILRSGDEIVDITNLEEYISLVVDATVKRGVTRQIEAFRSGFNQVFDITSLQIFTPSELDYLLCGRRELWEVETLAEHIKFDHGYNAKSPAIINLLEIMGELTADQQRAFCQFVTGAPRLPPGGLAVLNPKLTIVRKHSSTSSAAANGAGASETADDDLPSVMTCANYLKLPPYSTKEIMYKKLLYAINEGQGSFDLS

SEQ ID NO: 5 - DNA, 4524 bp, Brassica rapa
atggagaacagggggcagaaacgaatggaggatgtggaggagctacctgctgataagagagcttgtaactcacaggactctaggtcaagctcatctggtggctcgtctgttcagagccagtctcaagaagcagccaatggagcgagctcgggacacgaaaccactgacgctgatatggacacttcttcatcagattctccttctagtcattcagatggagagccagacaaggaggaggaggaggaggaggactacggatcttgcgattctgatgatgatgatgaagaaggtgaagatccgaggcacaaggcgcttcaggatgttcagtgggggagatcgtctgaggatcagcagaagttgagttctcttgtgacgagattgagtgaagaagtcgatccttctttgcagttgactggtcttacggagctgtgtgaggtcttgtctttctgtactgaagattcgctgtccaccgttatggccgatacgctttcccgggtgcttgttaagttggctaatcatgagagcaatgcagatattatgctgcttgctatcagagcggttacttacttgtctgatgtttatccgcggtctgtagcattccttgtgaaacatgagactctccctgctctttgccagagactacaggcaattgagtacttggacgttgctgagcagtgtttgcaagcacttgagaaaatatccaaagatgagccagtggcgtgcttgaatgctggagcaattaaggcagtgctttcgtatattgatttcttctcaactagcttacagagagtcgcagtttctactgtggtgaatatatgtaggaagctttcatctgagtctccctccccttttatggatgctgttccaattttatgcaatcttcttcagtatgaagatcgacagttggtggaaaatgtggctatttgcttaacaaaaatagcagatcaagttagcgagtcacctgaaatgttggatcaactatctagccatggtctgattcatcaatccatacatcttttaaacttgaatggccgcaccaccctatctcaacctgtttacaatggtgtgattggattgctaagaaaactatcttctggttcaattttagccttcagaacgttatatgaacttaacattggctacagactaaaagaaattatatccacgtatgacatttcccattcagtgtcttctacacatcccaacaatacatgttccaaccaggtgcatgaagtcctgaagttggtgattgagcttcttccatcttcgcctgtagaggataatcagctggcattggaaaaggaaagttttcttgttaatcagcccgatctcttgcaacaatttggagcagacatacttcctgttatgattcaggtgctaaaatctggagcgaacgtatatgttttttatggttgcctatcagcaatccacaagctgacttgcttgagtaagtcagtcgattttgtcgatttactgaagaatgcaaacattttaagtgttttggcgggcattttgtcaaggaaagttcatcatgtggttgttgtagcactacagattgctgaagcgcttcttgggaaatacagtgatgattttttgaattcgtttataaaggagggtgtttatttcgcaattgaagcgcttttaaactcggggcaacagaatcaaggatcagctgacggttcagaagagcatgttccgaaagagactgtgaaatgcttgtgccagtcttttgaaagatcgagttcctcttcttcacaaacttgtaagatcgagaaggattctgtctacattctcgcaacacgtatcaaggagagtttctttggacctgaggtattcgactctcagaaaggcttgacagatgttctccagaacctcaagcacttgtctgcagcacttgacgatttgatgactgaacctattgatgcacatgccctgcacgatgagaagttcttctcagtatggagccaaatcatggaaaggctgaatggaagggaatctgtgtccacatttgaatttacagagagtggagttgtgaaggcactgacaaattacctgtctaatagactccaccaaaggaaatttagcaaaggcgattcagaatgtgatagtttgccatttgttggtaacagatttgaagtgttcacaagatcactttggtctgatggcgaggcaacttcatccgtattaataaagaatctccaaaattccttatcttcattagagaactacccaattgtcctaagccagtttttgaagcaaaggaactcattcgcgactgttcccaatggacgtagcataagctatccaatcctaagagttcgttttgtcaaagcagagggggagacttgcttgcgtgattactcccaagacttggtcaccgttgacccactttgcttcttggatgctgtcgatcaatacatgtggcctaaagtgcagttagaacctttatattccgttgaagaaaaagatcaagctatggaatgtccatcttctcagctggagtcaacttctatatcttgtcaaggtgaaagctcaacccatatggagattgacagtcctaacgcatctcagttgcagggatctcaagaggaagaccaagagcagcttccagattcaggggaagataatacttcctcatctgaagaggaggatgcgttacctgaggaggatgcgttacctagacttttgtttcgtctagaagggcttgaactagaccgctctttgactgtataccaggctattctcttgcacaaactaaaatcaggaagtgaaactaccaacgattccaagctgagtggatcccacaccatcacgtatgaaagggccccacaacttgcagagtctgatgaaaatctgtttcctctcggatttatggacaatgacgagtatcacccgtttttatccttcttgtttgctcaaagacttgatttgcgccacaaagcaacaaatcctcctgcgtacgacatgttgtttctgctcaagagtctggagggcatgaacagatttctctttcacctgatttgtcatgaacggataaatgcttttggggaaggtaggctggagaatttggatgatctgagggtgcagcttcgtcctgtgccatatgctgaatttgttagtagtaagctaacagagaagctggagcagcagctgcgtgattcctttgctgtgtcaacctgcggtctaccaccgtggtttaatgatctaatgggttcatgcccttttctgtttagttttgaagtcaaaaccaaatacttccggctagcagcattcggttcgcagaaagtccatcatcatccacaacaccttagcagtgaagggcgcccagtaactggtagtttacctcgcaaaaagttcttagcttgccgtgaaaccattctagagtctgcttcaaaaatgatggagttgcacggcaaccagaaggtggtaattgaggttgagtacagtgaagaagtgggaactggtcttgggccaacgctggagttctacacacttgtcagtagagcgtttcaaaatccagaccttggcatgtggaggtgtgatcgtagttcctttgctggaaaaccaaaggaagactcaggatttttggtggctccttcgggactctttccacgaccttggtcagatacatcagctgctttcccagatgtgctacagaaatttgtgctcttagggacagtggtagcaaaggctctacatgatggacgagttttggacattcctttctccaaagccttctataaactgattatcggacaggagttgagttcatttgacatccacttcattgaccctgaactttgtaaaacactggtggaattgcaagctctgacacgtaggaaaaaggttttctcagaatcacaaactgatgcccgagcagccaagtgtgatttgagtttccgtggaacaaatattgaggatctttgtcttgaatttgtgctgcctggctacacagactatgttctcgctcttcattctgctaatgatatggtaaatttggataacctcgaggagtatatcaaggctattgtcaatgcaacaatatgtaacgggatccaaaaacaagtggaagcatttcggtctggatttaacaaagttttccctattgaacatcttgggatattcaatgaagaagaactggaaactctcttgtgtggagaacgagatctctttaatatgaatgaagtcttggatcacatcaagtttgatcatggatatacttctagcagcccaccagttgaaaatttgttggagattctgcatgagtttgacaaggatcaacaacgagcctttctgcagtttgtaacaggatgtcctcgtctacctcctgggggcttggcgtctctcaatcccaaactaacaattgtccgcaagcgtggtagcgattcttcagaaactgacttgccgagtgtgatgacatgcgctaattatctaaagcttccaccttactcttccaaagaaaagatgaaggagaagctaatttatgctataactgaaggccaaggttccttccatctctcttaa

SEQ ID NO: 6 - protein, 1507 aa, Brassica rapa
MENRGQKRMEDVEELPADKRACNSQDSRSSSSGGSSVQSQSQEAANGASSGHETTDADMDTSSSDSPSSHSDGEPDKEEEEEEDYGSCDSDDDDEEGEDPRHKALQDVQWGRSSEDQQKLSSLVTRLSEEVDPSLQLTGLTELCEVLSFCTEDSLSTVMADTLSRVLVKLANHESNADIMLLAIRAVTYLSDVYPRSVAFLVKHETLPALCQRLQAIEYLDVAEQCLQALEKISKDEPVACLNAGAIKAVLSYIDFFSTSLQRVAVSTVVNICRKLSSESPSPFMDAVPILCNLLQYEDRQLVENVAICLTKIADQVSESPEMLDQLSSHGLIHQSIHLLNLNGRTTLSQPVYNGVIGLLRKLSSGSILAFRTLYELNIGYRLKEIISTYDISHSVSSTHPNNTCSNQVHEVLKLVIELLPSSPVEDNQLALEKESFLVNQPDLLQQFGADILPVMIQVLKSGANVYVFYGCLSAIHKLTCLSKSVDFVDLLKNANILSVLAGILSRKVHHVVVVALQIAEALLGKYSDDFLNSFIKEGVYFAIEALLNSGQQNQGSADGSEEHVPKETVKCLCQSFERSSSSSSQTCKIEKDSVYILATRIKESFFGPEVFDSQKGLTDVLQNLKHLSAALDDLMTEPIDAHALHDEKFFSVWSQIMERLNGRESVSTFEFTESGVVKALTNYLSNRLHQRKFSKGDSECDSLPFVGNRFEVFTRSLWSDGEATSSVLIKNLQNSLSSLENYPIVLSQFLKQRNSFATVPNGRSISYPILRVRFVKAEGETCLRDYSQDLVTVDPLCFLDAVDQYMWPKVQLEPLYSVEEKDQAMECPSSQLESTSISCQGESSTHMEIDSPNASQLQGSQEEDQEQLPDSGEDNTSSSEEEDALPEEDALPRLLFRLEGLELDRSLTVYQAILLHKLKSGSETTNDSKLSGSHTITYERAPQLAESDENLFPLGFMDNDEYHPFLSFLFAQRLDLRHKATNPPAYDMLFLLKSLEGMNRFLFHLICHERINAFGEGRLENLDDLRVQLRPVPYAEFVSSKLTEKLEQQLRDSFAVSTCGLPPWFNDLMGSCPFLFSFEVKTKYFRLAAFGSQKVHHHPQHLSSEGRPVTGSLPRKKFLACRETILESASKMMELHGNQKVVIEVEYSEEVGTGLGPTLEFYTLVSRAFQNPDLGMWRCDRSSFAGKPKEDSGFLVAPSGLFPRPWSDTSAAFPDVLQKFVLLGTVVAKALHDGRVLDIPFSKAFYKLIIGQELSSFDIHFIDPELCKTLVELQALTRRKKVFSESQTDARAAKCDLSFRGTNIEDLCLEFVLPGYTDYVLALHSANDMVNLDNLEEYIKAIVNATICNGIQKQVEAFRSGFNKVFPIEHLGIFNEEELETLLCGERDLFNMNEVLDHIKFDHGYTSSSPPVENLLEILHEFDKDQQRAFLQFVTGCPRLPPGGLASLNPKLTIVRKRGSDSSETDLPSVMTCANYLKLPPYSSKEKMKEKLIYAITEGQGSFHLS

SEQ ID NO: 7 - DNA, 4446 bp, Brassica rapa
atggagaacagaggacagaaacgaatggaggttgtgggggagccacctgctgataagagagcttgcaactcacaagacttcacatctggcgcctcctctgctcaggctcaacaagccaatggtaacactgatgctgacatggacacttcttcctctgcctctccttcgagtcgttcagatggagaacaagacagggaggaggaggaggaggaggaatccgactacggatcatgcgattccgatgatgaggatccgaggaggagggtgcttcagcggtatcagagggggagatcaacaggagatcagctgaaactgaagtctctcgcgtcgaggttgagtgaagaaaacgatccttctctgcagttgactggtcttacggagctctgtgaagtgttgtctttctgtactgaggactctctgtccattgtgatggctgacttgctctcgcgtgtgcttgttaagttggctaagcatgagagcaatgcagatatcatgctgctcgcaatcagagcggttacttacttgtctgatgtttatccgcggtcggtagcgttccttgttaaacatgagaccattcctgctctctgccaaagactactgacgattgagtacttggatgttgctgagcagtgtttgcaagcacttgagaagatatccagagatcagccggtagcatgcttgaacgctggagcaattatggcagtgctttcgtatatcgatttcttttcaacaagcatacagagagtcgcagtttctactgtggtgaatatatgtaggaagcttccacctgagcctccctcgcctgtcatggatgctgttccagtattatgcaatcttcttcaatatgaagaccgacagttggtggagagtgtcgctatttgcttgacaaaaatagcagatcaagttagccagtcgcctgctatgttggatcaactatgtagccatggacttatccatcaatcaacacatcttttaaacttgaacagccgcacaaccctatctcaacctgtttacaacggcgtgattggattgctaagaaaactatcttctggttcaactttagctttcagaacattgtatgagcttaacattggctacagactaaaagaaatcatatccacctatgacatttctcattcagtttcttctacacagcccatccatccatgctccaaccaggtgcatgaagtcttgaagttggtgattgagcttcttccagcttcacctgttggggataatcagctggcattagaaaaggaaagttttcttgtcgatcagcctaatctcttgcaacaatttggagcagacatgcttcctgttatgactcaggtgctaaagtctggagctagcgtttatgtttcttatggttgcctatcagcaattcacaagctgacttgcttaagtaagtcagacgatcttgtcgagttactgaacaatgctaacatttcaagtgttttggcgggcattttttcaaggaaagatcatcatgtggtcgttgttgcactacagattgctgaagtgcttcttgagaaatacagagatgcttttttgaattcctttataaaagagggtgtttttttcgcaatcgcagcactcctaacttctgataggggacaacagatcaatccagtatccggtttcattcaaggatctgttccgaaagagattgtgaaatgcttgtgccagtcttttgaaggatcagtttcctcttcttcacaaacttgcaaggttggaaatgattctgtctacatcctcgcaacacgtatcaaggagagtttctttggacctgaggtattcgactctcagaaaggcttgacggatgtcctccagaacctcaagaatctgtcggcagaactcaacgatttggtgactgtacctgtcgatgcgcatgtcctgcatggtgagaggttcttctcaatatggaatcaaatcatggcaaggctgaaagagagggaatctgtgtccacttttgaatttactgagagtggagttgtgaaggctctggcaaattatctgtctaatggactctacgaaaggaaacttaacaaaggcgatcctgaatgtgatagtttaccacttgttggtaacagatttgaagtgttcacaagactactttggtctgatggcgaggcaactccgtccgctttaatacagaagctccaaaattccttatcttctttagaaaactacccaattgtcctgagccagtttttgaagcaaaggaactgtttcgctgctattccaaatggacgttgcataagttatccagtcctaagagttcgttttgctaaagcagagggggagacttgtctgcgtgattactctccaaactttgtcaccgttgacccactttgctacttggacgctgttagtcagtgcctgtggccccaagtgaatttggaacctttaaattctgtcgaagcgaaagatcaggctatagaatgtcaatcttcacagctgcagtcaacttcgatatcttgtcaaggtgaaagctcaagccatatggaaattgactgtcctaatgcatctcagctgcagggatctcaagaggaggaagaccaatatcaccttatagattcaggagaagagaattcttcctcatctaaagaagaggatgtgcgacctcgacttttgtttcgtctggaagggcttgagctagacccctctttgactgtttaccaggcaattctctcgcacaaactaaaatcagaaaatgagactaccaacgattcaaagcttagtggacaccacaccatcacttacgaaagagctccacagcttgcagtgtctcatgaaaatctgtttcccctcagatctatggacaacgacgagcatcacccgtttttatcctacttgtttgctcatagacttggtttgcgccacaaagggacaagtcctcctgagtatgccatattgtttctgctcaagagtctggagggcatgaacagatttctctttcagctgatttgtcatgaaaggattaatgcttttggggaaggtaggctggagagtttggatgatctaactgtgcaggtgcgtccggtgccatatgctgaatttgttagctctaagcttacagagaagttagagcagcagctgcgtgattcttttgctgtgtcaccgtgcggtctaccaccgtggtttaatgatctaatggcttcatgcccgtttctgtttagttttgaagtcaaatctaaatacttccgacttgcagcgttcggtccacagcaagtccataatcagccacagcaccttggtagttcaaatgttcatggtagtttacctcgtaaaaagtttttagcttgccgtgaaaagattctagagtctgctgcgaaaatgatggagttacacggcacccagaaggtggccgttgaggttgcgtacagtgaagaagtcggaactggccttgggccaacgctggagttctacacacttgtcagtagagcatttcaaaatccggatcttggtatgtggaggagtgatcctagctccttggctggaaagccaatggtacctccttcaggactctttccacgcccttggtcggctacatcagctgcttttccaggtgtgctgcagaagtttgttctcttggggacagtggtagccaaggctctacaagatggacgagtcttggacattcctttctctaaaaccttctataaactaattctcggacaggagttgagttcatttgacatccatttcgttgaccctgaactttgtaaaacactggtggaattgcaagctctggcacgtaggagaaaggttatctcagaatcacaaagtgatgtccgagcagctaagtgtgacttgagtttccgtggaacaaagattgaggacctttgtcttgatttttccctgcctggctacacggactatgttctctctcctcggtttgctaatgatatggtaaatttgggtaacctcgaggagtatgtaaaggctattgtcaatgccacagtatgtaatgggatcaaaaaacaagtggaagcgtttcggtctggatttaacaaagttttccctattgaacatcttaagatatttaatgaagaagaactggaaactttgttgtgtggagaacgagatctctttaatatgaatgaagtcttggaccacatcaagtttgatcatggttatacttctagcagcccaccagttcaaaatttgttggagattctgcatgagtttcacaaggagcaacagcgagcttttctgcaatttgtaacaggatgtcctcggctaccccctggcggtttggcgtctctcagtcccaaacttaccattgtccgcaagcacggtagtgattcatcagaaacagacctgcctagtgtgatgacctgcgccaattatctgaaacttccaccttactcttccaaagaaaagatgaaggagaagctgatctatgccataactgaagggcaaggttccttccatctctcttaa

SEQ ID NO: 8 - protein, 1481 aa, Brassica rapa
MENRGQKRMEVVGEPPADKRACNSQDFTSGASSAQAQQANGNTDADMDTSSSASPSSRSDGEQDREEEEEEESDYGSCDSDDEDPRRRVLQRYQRGRSTGDQLKLKSLASRLSEENDPSLQLTGLTELCEVLSFCTEDSLSIVMADLLSRVLVKLAKHESNADIMLLAIRAVTYLSDVYPRSVAFLVKHETIPALCQRLLTIEYLDVAEQCLQALEKISRDQPVACLNAGAIMAVLSYIDFFSTSIQRVAVSTVVNICRKLPPEPPSPVMDAVPVLCNLLQYEDRQLVESVAICLTKIADQVSQSPAMLDQLCSHGLIHQSTHLLNLNSRTTLSQPVYNGVIGLLRKLSSGSTLAFRTLYELNIGYRLKEIISTYDISHSVSSTQPIHPCSNQVHEVLKLVIELLPASPVGDNQLALEKESFLVDQPNLLQQFGADMLPVMTQVLKSGASVYVSYGCLSAIHKLTCLSKSDDLVELLNNANISSVLAGIFSRKDHHVVVVALQIAEVLLEKYRDAFLNSFIKEGVFFAIAALLTSDRGQQINPVSGFIQGSVPKEIVKCLCQSFEGSVSSSSQTCKVGNDSVYILATRIKESFFGPEVFDSQKGLTDVLQNLKNLSAELNDLVTVPVDAHVLHGERFFSIWNQIMARLKERESVSTFEFTESGVVKALANYLSNGLYERKLNKGDPECDSLPLVGNRFEVFTRLLWSDGEATPSALIQKLQNSLSSLENYPIVLSQFLKQRNCFAAIPNGRCISYPVLRVRFAKAEGETCLRDYSPNFVTVDPLCYLDAVSQCLWPQVNLEPLNSVEAKDQAIECQSSQLQSTSISCQGESSSHMEIDCPNASQLQGSQEEEDQYHLIDSGEENSSSSKEEDVRPRLLFRLEGLELDPSLTVYQAILSHKLKSENETTNDSKLSGHHTITYERAPQLAVSHENLFPLRSMDNDEHHPFLSYLFAHRLGLRHKGTSPPEYAILFLLKSLEGMNRFLFQLICHERINAFGEGRLESLDDLTVQVRPVPYAEFVSSKLTEKLEQQLRDSFAVSPCGLPPWFNDLMASCPFLFSFEVKSKYFRLAAFGPQQVHNQPQHLGSSNVHGSLPRKKFLACREKILESAAKMMELHGTQKVAVEVAYSEEVGTGLGPTLEFYTLVSRAFQNPDLGMWRSDPSSLAGKPMVPPSGLFPRPWSATSAAFPGVLQKFVLLGTVVAKALQDGRVLDIPFSKTFYKLILGQELSSFDIHFVDPELCKTLVELQALARRRKVISESQSDVRAAKCDLSFRGTKIEDLCLDFSLPGYTDYVLSPRFANDMVNLGNLEEYVKAIVNATVCNGIKKQVEAFRSGFNKVFPIEHLKIFNEEELETLLCGERDLFNMNEVLDHIKFDHGYTSSSPPVQNLLEILHEFHKEQQRAFLQFVTGCPRLPPGGLASLSPKLTIVRKHGSDSSETDLPSVMTCANYLKLPPYSSKEKMKEKLIYAITEGQGSFHLS

SEQ ID NO: 9 - DNA, 5553 bp, Solanum lycopersicum
atggaaactcggagccggaaacgaacggaggccacgtcatcagcgccttctgcttcttctccttcatcaggtcccaccacacgcgctgttaagaaagctcgttttaccacacgcgccgcctcaaactcgatctcaactcgttcccgactcacaaatcgttcccaagacctacaatcgatggactccacgaatgaatcatccgggtctggcagccgaaccaggcggggaaagaatcacgggttagatagaaataatccggagaagggtaaggagaaagagcacgaaattagggatagagacagagatatgggattgaacatggatactgatgggggtgatgaagatgataatgaaagtgaaggtggtgctgggattttgcaacataatttgacttcagcaagtagtgcacttcaaggactgttgagaaaattgggtgctggtttggatgatttactgccgagttcagcaatggtgtccgcttcctcgtcgcaacagaatgggcgtctgaagaagatattatcgggcttgagagctgacggggaagaagggaagcaaatagaggcattgacgcagctttgtgtgatgctttccattgggacagaagactctttgagcactttttcagtggactcttttgtacctgtcctggtggggctgcttaatcatatgagtaatcctgatattatgcttctcgcagctagggcgttaacccatttggttgatgttctgccatcttcttgtgctgctgttgtgcattatggagcggtttcatgttttgtagctcgcttactcacaattgaatacatggacttagctgagcagtctctacaagctttaaagaagatatctcaagaagatccaactgcttgtttgcaagcaggtgcactcatggctgtgctgtcgtatctcgatttcttttccactggtgttcagagagtagcactagcaactgctgctaatatgtgcaagaagctgccttcggatgctgctgactttgtgatggaagctgttccattgttgacgaatctccttcagtatcatgatgcaaaggtattagagcatgcttctatctgcttgacccggatagctgaagcatttgcatcatctccagaaaagctagatgaactctgtaatcacggacttgtcacacaggctgcctccctcatctcaaccagtaattctggaggtggtcaggcttcactcagcacggaaacttacacaggcttgatccggcttctttgtacttgtgccagtggctcaccattaggggctaaaaccttgatgatgcttggtatcagtgggatcctcaaggacattttatcagcctctgtctctatttcacctgccatgagcagacctgcggagcagatttttgagattgtgaatcttgcaaatgaactacttcctccgctgcctcaaggaattatctctcttcctgttagcacaaatttgttcattagaggtccttttacgcggaaatcctctgctagtggttctagcaaacaggaggatcttaatgcatcttctcaggaggtatcagctcatgagaaactattgaatgatcaacctgaacttctgcaacaatttggaatggatctccttcctgttctgatacagacatatggatccagtgtaaatacagcagcacgccacaaatgcctctcagttattggaaaacttatgtatttcagtaatgcagatatgattcaatctttaactaatgacactaacttgtcaagtttcttggctggggttttggcgtggaaggatccccaagtattggtccccgctcttcaaatagcagagattctaatggagaagctccctggagtttttggcaagatgtttgtccgggaaggtgttgttcatgctgtagatgccttgatgttgtctgggtctcatgtttctgctcctccccatccaacacgtgctgagaaagagaaacataatagacgccgtagcactaattccaatacagatgcaatttctgttgaagatcttacaagtccagttccaagtactggatctctgccaaattcaatggaaattcggaccgttaattctagcctccggatgtcagtcagtacatgtgcaaaagctttcaaggataaatacttcccatcagattctgaggctgctgaagctggtgtcacggatgatcttatacgattgaagaatctctgcatgaagttgaatgctggtattgatgagcagatagctaaacctaaaggaaaatccaaaacatttggtcctcagcttggggatagctatgttggaaaagaagaaaacttggctgaagtgatagctgccatgatgggggaactcagcaaaggggatggtgtttcaacttttgagttcagtggaagtggagttgttgcttctttgctgaaatattttacgtttgcgtacttttctaaggaaagaatctctgatactagtatgtctaagcttcgacaacaagcaatcagaagatacaagtcttttattgcagttgcccttcctgctggtgttgatggtggaaatatggttcccatgactgttctggtccaaaagcttcaaaatgctctatgttcattggagcgttttcctgttgtattgagtcatagttccagatcatcgacaggaaatgcacgtctttcttcaggtttaagtgttttgtctcagccttttaagctgcgcctttgcagagctcaaggagagaaaaccctccgtgactactcttcaaatgttttgctgattgatcctttggcaagtttagtagctattgaagaattcctttgggcccgagttgggagacctgaggctgaacagaaggcatctgctactggtggaaactctgggtctgggactatacctgctggaggcagtgcgtcatctccatctatgtccactcctgcctctgcatctcgtcgtcattctgctcgatcaaggtcagcagttaatattaatgaaagtgatggaagctcttcaaagggcaaaggtaaagcggttttgaagcctgctcaaaaagatcgcaggggaattcgatcaagagatcctgttaaaataagagctgccttggagaaggccttaagagaggagcctgttgatggggagactagttcagaggatgacgagctgcatccttctctcattgaacttgatgatgctttggtgattgaggatgatatgttcgatgaagatgaagatgaccatgatgatgtgctgagggatgatccttttcctgtctgcatggcagatgaagtgcatgatgttaaattgggagactcttcggaggatagcccttttgcacagacaccaactggcagcaatacaaatgctggtggtggttctgggagcagaattgcttctgctcggggatctgattccgttgagttcagaagtaggaactcgtatggttcaaggggggcaatgtcatttgctgctgctgccatggctggtctttcatctgctagtgttagaggtgtgaggggcgctagagatcgacatgggcatcctctactcagctctggtgatccaccaaaactaatattttctgttggtgggaagccgcttaataggcagttgactatctaccaggctatccagcggcagcttgttctagacgaggatgatgatgagagatatggtggcaatgattttgtatctggtgacggcagtagggtttggagtgatatttacacgatcacataccagagggcagacaaccaagctgagaggtcaagtgggtctgggagttcaatttccaagtctatgaaaaccagttcttcaacaagttccggtgctgatccttcattggttcaagcatcattgttagatagtatattgcagggagaacttccttgtgatctggagaaaagtaaccctacttacagtattttgtacctcttacgtgtattggaggcgctgaatcagcttgccccccgtttgagagtcctgtccatgattgatgatttctctgaaggaaaaatttctagtctagatgagctcggtactacgggtatcaaaatcccttctgaggaatttgtcaatagtaagctcactccgaaattggcacgacagatccaggatgctcttgcactttgtagtggatctcttccatcttggtgttaccagttgaccaaggcctgcccatttctttttccatttgagactcggcgccagtacttctattcaactgcttttgggttgtcacgtgctttatataggctgcagcaacagcaaggtgctgatggtaatgggtctactcatgagagagcagttagggttggcagattacagcgccagaaagttcgtgtctcaaggaaccgcattctggattctgctgcaaaagtaatggagatgtactctagccaaaaagctgttcttgaagttgaatattttggtgaagttggtactggcctgggtcctacacttgagttttatacccttataagtcacgatctacagaaacttggacttggaatgtggagatctggtttatcattaacttcaaatgaacattctgtggaagttcatatcgataataaattaagtagaagtgacggagatcttgtccaagcacctcttggattattcccacgtccctggtcaccacatactggtactgttgatggaggtcaattctataaagcaattgaatatttccgcttgcttggacgtgttatggcgaaagctcttcaagatggacggcttttggaccttccactgtccatggccttctataagctcgttcttggtcaagaacttgatttgtatgatattctttcttttgacaccgaattggggaagactttgcaagagttgcaagccctcgtcagtcgaaagcaatatatagaatcaataaaagatcagaacctggacgagtcttatgacatgcattttcgtgggactccagttgaggatctttgtttagatttcacacttcctggctatcctgaatatattcttaaagcaggcgacgagaatgtgagtcgcgatatcgtggattttaacttggaggagtatatttctttggtagttgatgctactgtgaaaactggaatcaggcagcaaatggaggcttttagatctggcttcaatcaggttttcgacttttcagctctgcaaatattctctccttcagagttagactatctattatgtggccgtagagagctgtggaagcctgagacgctagtagatcacataaaattcgatcatggattcacatccaagagtcctcctattattcatttactagagattatgggagagttcacacctgagcagcaacgagcattctgccagtttgttactggtgctcctcggctccccgcaggtggtcttgcttctctgaatcctaagttgacaattgtgaggaagcattcatctagtgctggcaatgcagcacagaacagtaatgccccatcagaatctgcagatgaagacctacccagtgtgatgacatgtgctaattacttgaaactccctccctattctactaaggagatcatgtccaagaaattactctatgccattaatgaaggtcaaggatcgtttgatttgtcataa

SEQ ID NO: 10 - protein, 1850 aa, Solanum lycopersicum
METRSRKRTEATSSAPSASSPSSGPTTRAVKKARFTTRAASNSISTRSRLTNRSQDLQSMDSTNESSGSGSRTRRGKNHGLDRNNPEKGKEKEHEIRDRDRDMGLNMDTDGGDEDDNESEGGAGILQHNLTSASSALQGLLRKLGAGLDDLLPSSAMVSASSSQQNGRLKKILSGLRADGEEGKQIEALTQLCVMLSIGTEDSLSTFSVDSFVPVLVGLLNHMSNPDIMLLAARALTHLVDVLPSSCAAVVHYGAVSCFVARLLTIEYMDLAEQSLQALKKISQEDPTACLQAGALMAVLSYLDFFSTGVQRVALATAANMCKKLPSDAADFVMEAVPLLTNLLQYHDAKVLEHASICLTRIAEAFASSPEKLDELCNHGLVTQAASLISTSNSGGGQASLSTETYTGLIRLLCTCASGSPLGAKTLMMLGISGILKDILSASVSISPAMSRPAEQIFEIVNLANELLPPLPQGIISLPVSTNLFIRGPFTRKSSASGSSKQEDLNASSQEVSAHEKLLNDQPELLQQFGMDLLPVLIQTYGSSVNTAARHKCLSVIGKLMYFSNADMIQSLTNDTNLSSFLAGVLAWKDPQVLVPALQIAEILMEKLPGVFGKMFVREGVVHAVDALMLSGSHVSAPPHPTRAEKEKHNRRRSTNSNTDAISVEDLTSPVPSTGSLPNSMEIRTVNSSLRMSVSTCAKAFKDKYFPSDSEAAEAGVTDDLIRLKNLCMKLNAGIDEQIAKPKGKSKTFGPQLGDSYVGKEENLAEVIAAMMGELSKGDGVSTFEFSGSGVVASLLKYFTFAYFSKERISDTSMSKLRQQAIRRYKSFIAVALPAGVDGGNMVPMTVLVQKLQNALCSLERFPVVLSHSSRSSTGNARLSSGLSVLSQPFKLRLCRAQGEKTLRDYSSNVLLIDPLASLVAIEEFLWARVGRPEAEQKASATGGNSGSGTIPAGGSASSPSMSTPASASRRHSARSRSAVNINESDGSSSKGKGKAVLKPAQKDRRGIRSRDPVKIRAALEKALREEPVDGETSSEDDELHPSLIELDDALVIEDDMFDEDEDDHDDVLRDDPFPVCMADEVHDVKLGDSSEDSPFAQTPTGSNTNAGGGSGSRIASARGSDSVEFRSRNSYGSRGAMSFAAAAMAGLSSASVRGVRGARDRHGHPLLSSGDPPKLIFSVGGKPLNRQLTIYQAIQRQLVLDEDDDERYGGNDFVSGDGSRVWSDIYTITYQRADNQAERSSGSGSSISKSMKTSSSTSSGADPSLVQASLLDSILQGELPCDLEKSNPTYSILYLLRVLEALNQLAPRLRVLSMIDDFSEGKISSLDELGTTGIKIPSEEFVNSKLTPKLARQIQDALALCSGSLPSWCYQLTKACPFLFPFETRRQYFYSTAFGLSRALYRLQQQQGADGNGSTHERAVRVGRLQRQKVRVSRNRILDSAAKVMEMYSSQKAVLEVEYFGEVGTGLGPTLEFYTLISHDLQKLGLGMWRSGLSLTSNEHSVEVHIDNKLSRSDGDLVQAPLGLFPRPWSPHTGTVDGGQFYKAIEYFRLLGRVMAKALQDGRLLDLPLSMAFYKLVLGQELDLYDILSFDTELGKTLQELQALVSRKQYIESIKDQNLDESYDMHFRGTPVEDLCLDFTLPGYPEYILKAGDENVSRDIVDFNLEEYISLVVDATVKTGIRQQMEAFRSGFNQVFDFSALQIFSPSELDYLLCGRRELWKPETLVDHIKFDHGFTSKSPPIIHLLEIMGEFTPEQQRAFCQFVTGAPRLPAGGLASLNPKLTIVRKHSSSAGNAAQNSNAPSESADEDLPSVMTCANYLKLPPYSTKEIMSKKLLYAINEGQGSFDLS

SEQ ID NO: 11 - DNA, 3612 bp, Oryza sativa
atggagtgccccaaggagtgcctcagccacggcgtgccagccgccgtgctgcagttcttcgacttcttctcgatgcacaagcagaagctggtgctcaagatcgtcgccaacgtcttgggcgacttcagcgcgaaggatgcggccaaggccatggaggccgcgcccgttctgtgcaacctcctgcaatccactgacaagacgatactcgactccgccgtttcttgcttggttttggtctctgatggtgcttgcgacagtgcccaacacatggaaaagctttacgagcttaatgcagtccaagcgacgatgaggttgatggagaacgacgggtggaagagcctcagcgatgagactttatctggcatccttggtcttctcaaagacctagcttctctctcagcaagggctgtaaagtctctttttgagttaaacatttgtgatttgctcaagcagatgataacatactacacctcgtcgcacagtgatcacaataaggtgcagacgcttgtagagctcatttattatcttatgccacctcttgaaatgtgtgaccatcgtaccgaactaatcattgcaaagaagaatgtcatcacagaacaaagtggatacatccaacagcttgctagcatccttacttttataatacaggttgcgaaatctgctgcactatcatcaatttgctacagttgtgttgttgtcatcagaaacattgttgaattaagcacaccttcttccttggtggaggtacagaagacagtaaacctgtcaagcttacttgctggctggttggcccggaagaaccgccatatcatattccaaacgctcaacgtttcgaagacccttctgagaaaagaccagaaattcttctttgagaccttcatcagggagggtctaaagcatgcaattgatgcaatactaacacaggaaaaaggaaagagccgcttgccagaaagttgcctttgttttgatttagacttggagacctcgacagatgatgcatgcaggattaataatggtgctatcctgaaactagcggaggagataaagaaaaacttcttggtaaaggttgccaagtctcctcacaagtttgggtgtgcttttaaaagcataaaggaatttttttctcgtttgaattgtcatgccacggcacccccagctaaagatcaggatctctgcaagcagttgtctgatttttcaaggcaattattatcggatgaactgccaagtacttctacttttgagtttgtgcagagtggatctatcaaacatttggcaggttatctttccaatgggacatactttaattcaaatctcaggaattgccaggacttgataggggagcttaaggaggtgaaaatccggctgcagaagttcacgcacttggctctcagcgtggacaatgaaagctcggtgaagccacttgagattttggtggagaaactgatagatgcgttgcatgtgtggtatgacagtttccctgtaatcctggctgatgaacagtgcacacgtgagagcaccatgattcctctgagggattcaggaactgaggaaccaatgtcactatatataaaattttcgagatcagccagggaggaggagttggaggattatggtggagttctccctgttgatctttcttcgacacctgaatccattgaagaggtcctgttgcctgagatctgtaaaagaactggcaatgaaacttcatacaaggaaaacactcaagaagcaaatgggagcagaaaatctgttgggctcagaaatggtgacgggcacaagttctcaagattgaaattctcttacaaaggaacacaactccagtcatctacaccactttttgagtcaatcctccgctcaatgcatgaaggagaaaccgatctccagattgacccatctttttgggataaagaacacaagatagtatacagaagaagaaacaaaagcaagaaaatatcttcccatagttcctacaatattcagttgtgccgtgtgcatgaaaaacttgaaatgtcattgcttaaggacccctttttctccaccatactcactggcaagcttcctggtgatctggatgaatctgatccatcatataacttcctgttcatgctgaaagtcctcgaagggctcaaccgtttttcatatcatctatcaatggatgataagttatgcaaatttgctgaaggctgcctccaagagtttgatgaccttaaggtggcaatttgtccaattccacgggatcagttcgtgagcagtctactgacaaataagttagagcagcaaatgcaagatagcttgtttggggatggcttgataccctcgtggtgtatctatttggttgaaacttgcccgttcttgttgtcattcgaagctcgatggaagtatttctgcctgacggcacatcactcattcatgacagatgaggctagcagttcaacagaaactaagaagtacagcgtaacacggagcaaaatccttgaagatgcttcatcgatgttgaacaaacatggatcagacaccaaattcattgaggtggaatttgatggagaggttgggaccggtcgaggcccaaccttcgaattctataccacagttagtcatgaactacagagagtgggtcttggaatgtggagaggagacgacaccagccaagaatgcgaagctggttttgtccatgccccttttggtctctttccacagccatggtcctcagcaaacacttcatctcaagggatcagtttgtccaatgtggtacaaaaattcaagcttcttgggcatcttgtagcaagagcagttttggatggaagggttctggatattcctctctcgaaagcattttacaagatcatgcttgagcaggaccttgatatttatgacattccatcatttgatcccaagttgggcaagactgttatggagtttcaagcacttgttaaaaggaagaagttcctggaggaaagggcatccaatccagcagctgatttgtcctataaaaacgtgcgattggaggatttatgtcttgactttacccttcctggaaatccggaatatgaacttgtccctggaggttcagagaagatggtgacacttgacaatttggaggagtatgtgtcttcaattgttgatgcaaccttgaaaagtgggatatccaatcaaatagaagctttcaaggctggaattaacaaggtttttgctcttaagactcttcggttgttcagtgaggatgagatggagcgtatactatgtggcgaacaagattcttgggcttcgaacaaacttgaggatcacatcaattttgattatggatatgatgcgaacagtgcatcagtaattagtttcctggagatcttgcgggagtttggaagagaggaccagcgggcgttcttgcattttacgactggagctcctcagctcccacttggtggcctagcttcgctcgatcctaagctcaccgtagtgcgaaagcaatgtgatggcaaagtagacaacgaattaccgagtgtcaatacttgccggcatttcttcaagcttccaccgtactcctctaaggagattatgagacagaagctcaaatatgctatcaaggagggtttaggctccttccaattatcatga

SEQ ID NO: 12 - protein, 1203 aa, Oryza sativa
MECPKECLSHGVPAAVLQFFDFFSMHKQKLVLKIVANVLGDFSAKDAAKAMEAAPVLCNLLQSTDKTILDSAVSCLVLVSDGACDSAQHMEKLYELNAVQATMRLMENDGWKSLSDETLSGILGLLKDLASLSARAVKSLFELNICDLLKQMITYYTSSHSDHNKVQTLVELIYYLMPPLEMCDHRTELIIAKKNVITEQSGYIQQLASILTFIIQVAKSAALSSICYSCVVVIRNIVELSTPSSLVEVQKTVNLSSLLAGWLARKNRHIIFQTLNVSKTLLRKDQKFFFETFIREGLKHAIDAILTQEKGKSRLPESCLCFDLDLETSTDDACRINNGAILKLAEEIKKNFLVKVAKSPHKFGCAFKSIKEFFSRLNCHATAPPAKDQDLCKQLSDFSRQLLSDELPSTSTFEFVQSGSIKHLAGYLSNGTYFNSNLRNCQDLIGELKEVKIRLQKFTHLALSVDNESSVKPLEILVEKLIDALHVWYDSFPVILADEQCTRESTMIPLRDSGTEEPMSLYIKFSRSAREEELEDYGGVLPVDLSSTPESIEEVLLPEICKRTGNETSYKENTQEANGSRKSVGLRNGDGHKFSRLKFSYKGTQLQSSTPLFESILRSMHEGETDLQIDPSFWDKEHKIVYRRRNKSKKISSHSSYNIQLCRVHEKLEMSLLKDPFFSTILTGKLPGDLDESDPSYNFLFMLKVLEGLNRFSYHLSMDDKLCKFAEGCLQEFDDLKVAICPIPRDQFVSSLLTNKLEQQMQDSLFGDGLIPSWCIYLVETCPFLLSFEARWKYFCLTAHHSFMTDEASSSTETKKYSVTRSKILEDASSMLNKHGSDTKFIEVEFDGEVGTGRGPTFEFYTTVSHELQRVGLGMWRGDDTSQECEAGFVHAPFGLFPQPWSSANTSSQGISLSNVVQKFKLLGHLVARAVLDGRVLDIPLSKAFYKIMLEQDLDIYDIPSFDPKLGKTVMEFQALVKRKKFLEERASNPAADLSYKNVRLEDLCLDFTLPGNPEYELVPGGSEKMVTLDNLEEYVSSIVDATLKSGISNQIEAFKAGINKVFALKTLRLFSEDEMERILCGEQDSWASNKLEDHINFDYGYDANSASVISFLEILREFGREDQRAFLHFTTGAPQLPLGGLASLDPKLTVVRKQCDGKVDNELPSVNTCRHFFKLPPYSSKEIMRQKLKYAIKEGLGSFQLS